European Patent Application EP 4 349 861 A1, published April 10, 2024. Title: BISPECIFIC BINDING MOLECULE BINDING TO VEGF AND ANG2 AND USE THEREOF. Applicant: INNOVENT BIOLOGICS (SUZHOU) CO., LTD. The sequence listing filed with the application follows.

SEQUENCE LISTING (42 sequences)

SEQ ID NO: 1 - protein, 10 aa, Artificial
  Synthetic construct
GFNLDYYPIG

SEQ ID NO: 2 - protein, 16 aa, Artificial
  Synthetic construct
CISSVGSTNYADSVKG

SEQ ID NO: 3 - protein, 15 aa, Artificial
  Synthetic construct
DPLCSALILPPPFLS

SEQ ID NO: 4 - protein, 123 aa, Artificial
  Synthetic construct
QLQLVESGGGLVQPGGSLRLSCAASGFNLDYYPIGWFRQAPGKEREGVSCISSVGSTNYADSVKGRFTISRDNAKNTVYLQMNSLKPEDTAVYYCAADPLCSALILPPPFLSWGQGTQVTVSS

SEQ ID NO: 5 - protein, 123 aa, Artificial
  Synthetic construct
EVQLLESGGGLVQPGGSLRLSCAASGFNLDYYPIGWFRQAPGKGLEGVSCISSVGSTNYADSVKGRFTISRDNSKNTVYLQMNSLRAEDTAVYYCAADPLCSALILPPPFLSWGQGTQVTVSS

SEQ ID NO: 6 - protein, 10 aa, Artificial
  Synthetic construct
GSIFSINAMG

SEQ ID NO: 7 - protein, 16 aa, Artificial
  Synthetic construct
TMIGGSSTFYADSVNG

SEQ ID NO: 8 - protein, 17 aa, Artificial
  Synthetic construct
DVTGRSGTSIWNKRDDY

SEQ ID NO: 9 - protein, 125 aa, Artificial
  Synthetic construct
QVQLEESGGGLVQPGGSLRLSCVASGSIFSINAMGWHRQAPGSQRELVATMIGGSSTFYADSVNGRFTISRDNAKNTVYLQMNSLKLEDTAVYYCYADVTGRSGTSIWNKRDDYWGQGTLVTVSS

SEQ ID NO: 10 - protein, 16 aa, Artificial
  Synthetic construct
TMIGGSSTFYAESVQG

SEQ ID NO: 11 - protein, 125 aa, Artificial
  Synthetic construct
EVQLLESGGGLVQPGGSLRLSCAASGSIFSINAMGWHRQAPGKQRELVATMIGGSSTFYAESVQGRFTISRDNSKNTVYLQMNSLRAEDTAVYYCYADVTGRSGTSIWNKRDDYWGQGTQVTVSS

SEQ ID NO: 12 - protein, 125 aa, Artificial
  Synthetic construct
DVQLVESGGGLVQPGGSLRLSCAASGRTFSSYSMGWFRQAPGKEREFVVAISKGGYKYDAVSLEGRFTISRDNAKNTVYLQINSLRPEDTAVYYCASSRAYGSSRLRLADTYEYWGQGTLVTVSS

SEQ ID NO: 13 - protein, 453 aa, Artificial
  Synthetic construct
EVQLVESGGGLVQPGGSLRLSCAASGYDFTHYGMNWVRQAPGKGLEWVGWINTYTGEPTYAADFKRRFTFSLDTSKSTAYLQMNSLRAEDTAVYYCAKYPYYYGTSHWYFDVWGQGTLVTVSSASTKGPSVFPLAPSSKSTSGGTAALGCLVKDYFPEPVTVSWNSGALTSGVHTFPAVLQSSGLYSLSSVVTVPSSSLGTQTYICNVNHKPSNTKVDKKVEPKSCDKTHTCPPCPAPEAAGGPSVFLFPPKPKDTLMASRTPEVTCVVVDVSHEDPEVKFNWYVDGVEVHNAKTKPREEQYNSTYRVVSVLTVLAQDWLNGKEYKCKVSNKALGAPIEKTISKAKGQPREPQVYTLPPCRDELTKNQVSLWCLVKGFYPSDIAVEWESNGQPENNYKTTPPVLDSDGSFFLYSKLTVDKSRWQQGNVFSCSVMHEALHNAYTQKSLSLSPGK

SEQ ID NO: 14 - protein, 463 aa, Artificial
  Synthetic construct
QVQLVQSGAEVKKPGASVKVSCKASGYTFTGYYMHWVRQAPGQGLEWMGWINPNSGGTNYAQKFQGRVTMTRDTSISTAYMELSRLRSDDTAVYYCARSPNPYYYDSSGYYYPGAFDIWGQGTMVTVSSASVAAPSVFIFPPSDEQLKSGTASVVCLLNNFYPREAKVQWKVDNALQSGNSQESVTEQDSKDSTYSLSSTLTLSKADYEKHKVYACEVTHQGLSSPVTKSFNRGECDKTHTCPPCPAPEAAGGPSVFLFPPKPKDTLMASRTPEVTCVVVDVSHEDPEVKFNWYVDGVEVHNAKTKPREEQYNSTYRVVSVLTVLAQDWLNGKEYKCKVSNKALGAPIEKTISKAKGQPREPQVCTLPPSRDELTKNQVSLSCAVKGFYPSDIAVEWESNGQPENNYKTTPPVLDSDGSFFLVSKLTVDKSRWQQGNVFSCSVMHEALHNAYTQKSLSLSPGK

SEQ ID NO: 15 - protein, 387 aa, Artificial
  Synthetic construct
DVQLVESGGGLVQPGGSLRLSCAASGRTFSSYSMGWFRQAPGKEREFVVAISKGGYKYDAVSLEGRFTISRDNAKNTVYLQINSLRPEDTAVYYCASSRAYGSSRLRLADTYEYWGQGTLVTVSSGGGGSGGGSEVQLVESGGGLVQPGNSLRLSCAASGFTFSSFGMSWVRQAPGRGLEWVSSISGSGSDTLYADSVKGRFTISRDNAKTTLYLQMNSLRPEDTAVYYCTIGGSLSRSSQGTLVTVSSGGGGSGGGSEVQLVESGGGLVQPGGSLRLSCAVSGITLDDYAIGWFRQAPGKEREGVSAIRSSGGSTYYADSVKGRFTISSDNSKNTVYLQMNSLRPEDTAVYYCAAVPAGRLRYGEQWYPIYEYDAWGQGTLVTVSS

SEQ ID NO: 16 - protein, 10 aa, Artificial
  Synthetic construct
GFALDYYAIG

SEQ ID NO: 17 - protein, 17 aa, Artificial
  Synthetic construct
CISSGDGSTYYADSVKG

SEQ ID NO: 18 - protein, 19 aa, Artificial
  Synthetic construct
DSRGDDVACEGLRRNEYDY

SEQ ID NO: 19 - protein, 128 aa, Artificial
  Synthetic construct
QVQLVESGGGLVQPGGSLRLSCAASGFALDYYAIGWFRQAPGKEREGVSCISSGDGSTYYADSVKGRFTISRDNAKNTVYLQMNSLKPEDTAVYYCATDSRGDDVACEGLRRNEYDYWGQGTQVTVSS

SEQ ID NO: 20 - protein, 17 aa, Artificial
  Synthetic construct
CISSGEGSTYYADSVKG

SEQ ID NO: 21 - protein, 128 aa, Artificial
  Synthetic construct
EVQLLESGGGLVQPGGSLRLSCAASGFALDYYAIGWFRQAPGKGLEGVSCISSGEGSTYYADSVKGRFTISRDNSKNTVYLQMNSLRAEDTAVYYCATDSRGDDVACEGLRRNEYDYWGQGTLVTVSS

SEQ ID NO: 22 - protein, 398 aa, Artificial
  Synthetic construct
EVQLLESGGGLVQPGGSLRLSCAASGSIFSINAMGWHRQAPGKQRELVATMIGGSSTFYAESVQGRFTISRDNSKNTVYLQMNSLRAEDTAVYYCYADVTGRSGTSIWNKRDDYWGQGTQVTVSSGGGGSGGGGSEVQLLESGGGLVQPGGSLRLSCAASGSIFSINAMGWHRQAPGKQRELVATMIGGSSTFYAESVQGRFTISRDNSKNTVYLQMNSLRAEDTAVYYCYADVTGRSGTSIWNKRDDYWGQGTQVTVSSGGGGSGGGGSEVQLLESGGGLVQPGGSLRLSCAASGFALDYYAIGWFRQAPGKGLEGVSCISSGEGSTYYADSVKGRFTISRDNSKNTVYLQMNSLRAEDTAVYYCATDSRGDDVACEGLRRNEYDYWGQGTLVTVSS

SEQ ID NO: 23 - protein, 5 aa, Artificial
  Synthetic construct
  REPEAT (1)..(5): repeat 1 to 4 times
GGGGS

SEQ ID NO: 24 - protein, 574 aa, Artificial
  Synthetic construct
SDTGRPFVEMYSEIPEIIHMTEGRELVIPCRVTSPNITVTLKKFPLDTLIPDGKRIIWDSRKGFIISNATYKEIGLLTCEATVNGHLYKTNYLTHRQTNTIIDVVLSPSHGIELSVGEKLVLNCTARTELNVGIDFNWEYPSSKHQHKKLVNRDLKTQSGSEMKKFLSTLTIDGVTRSDQGLYTCAASSGLMTKKNSTFVRVHEKDKTHTCPPCPAPELLGGPSVFLFPPKPKDTLMISRTPEVTCVVVDVSHEDPEVKFNWYVDGVEVHNAKTKPREEQYNSTYRVVSVLTVLHQDWLNGKEYKCKVSNKALPAPIEKTISKAKGQPREPQVYTLPPSRDELTKNQVSLTCLVKGFYPSDIAVEWESNGQPENNYKTTPPVLDSDGSFFLYSKLTVDKSRWQQGNVFSCSVMHEALHNHYTQKSLSLSPGGGGGSGGGGSGGGGSEVQLLESGGGLVQPGGSLRLSCAASGFALDYYAIGWFRQAPGKGLEGVSCISSGEGSTYYADSVKGRFTISRDNSKNTVYLQMNSLRAEDTAVYYCATDSRGDDVACEGLRRNEYDYWGQGTLVTVSS

SEQ ID NO: 25 - protein, 431 aa, Artificial
  Synthetic construct
SDTGRPFVEMYSEIPEIIHMTEGRELVIPCRVTSPNITVTLKKFPLDTLIPDGKRIIWDSRKGFIISNATYKEIGLLTCEATVNGHLYKTNYLTHRQTNTIIDVVLSPSHGIELSVGEKLVLNCTARTELNVGIDFNWEYPSSKHQHKKLVNRDLKTQSGSEMKKFLSTLTIDGVTRSDQGLYTCAASSGLMTKKNSTFVRVHEKDKTHTCPPCPAPELLGGPSVFLFPPKPKDTLMISRTPEVTCVVVDVSHEDPEVKFNWYVDGVEVHNAKTKPREEQYNSTYRVVSVLTVLHQDWLNGKEYKCKVSNKALPAPIEKTISKAKGQPREPQVYTLPPSRDELTKNQVSLTCLVKGFYPSDIAVEWESNGQPENNYKTTPPVLDSDGSFFLYSKLTVDKSRWQQGNVFSCSVMHEALHNHYTQKSLSLSPG

SEQ ID NO: 26 - protein, 205 aa, Artificial
  Synthetic construct
SDTGRPFVEMYSEIPEIIHMTEGRELVIPCRVTSPNITVTLKKFPLDTLIPDGKRIIWDSRKGFIISNATYKEIGLLTCEATVNGHLYKTNYLTHRQTNTIIDVVLSPSHGIELSVGEKLVLNCTARTELNVGIDFNWEYPSSKHQHKKLVNRDLKTQSGSEMKKFLSTLTIDGVTRSDQGLYTCAASSGLMTKKNSTFVRVHEK

SEQ ID NO: 27 - protein, 226 aa, Artificial
  Synthetic construct
DKTHTCPPCPAPELLGGPSVFLFPPKPKDTLMISRTPEVTCVVVDVSHEDPEVKFNWYVDGVEVHNAKTKPREEQYNSTYRVVSVLTVLHQDWLNGKEYKCKVSNKALPAPIEKTISKAKGQPREPQVYTLPPSRDELTKNQVSLTCLVKGFYPSDIAVEWESNGQPENNYKTTPPVLDSDGSFFLYSKLTVDKSRWQQGNVFSCSVMHEALHNHYTQKSLSLSPG

SEQ ID NO: 28 - protein, 393 aa, Artificial
  Synthetic construct
DIQLTQSPSSLSASVGDRVTITCSASQDISNYLNWYQQKPGKAPKVLIYFTSSLHSGVPSRFSGSGSGTDFTLTISSLQPEDFATYYCQQYSTVPWTFGCGTKVEIKGGGGSGGGGSGGGGSGGGGSEVQLVESGGGLVQPGGSLRLSCAASGYDFTHYGMNWVRQAPGKCLEWVGWINTYTGEPTYAADFKRRFTFSLDTSKSTAYLQMNSLRAEDTAVYYCAKYPYYYGTSHWYFDVWGQGTLVTVSSGGGGSGGGGSGGGGSEVQLLESGGGLVQPGGSLRLSCAASGFALDYYAIGWFRQAPGKGLEGVSCISSGEGSTYYADSVKGRFTISRDNSKNTVYLQMNSLRAEDTAVYYCATDSRGDDVACEGLRRNEYDYWGQGTLVTVSS

SEQ ID NO: 29 - protein, 250 aa, Artificial
  Synthetic construct
DIQLTQSPSSLSASVGDRVTITCSASQDISNYLNWYQQKPGKAPKVLIYFTSSLHSGVPSRFSGSGSGTDFTLTISSLQPEDFATYYCQQYSTVPWTFGCGTKVEIKGGGGSGGGGSGGGGSGGGGSEVQLVESGGGLVQPGGSLRLSCAASGYDFTHYGMNWVRQAPGKCLEWVGWINTYTGEPTYAADFKRRFTFSLDTSKSTAYLQMNSLRAEDTAVYYCAKYPYYYGTSHWYFDVWGQGTLVTVSS

SEQ ID NO: 30 - protein, 107 aa, Artificial
  Synthetic construct
DIQLTQSPSSLSASVGDRVTITCSASQDISNYLNWYQQKPGKAPKVLIYFTSSLHSGVPSRFSGSGSGTDFTLTISSLQPEDFATYYCQQYSTVPWTFGCGTKVEIK

SEQ ID NO: 31 - protein, 8 aa, Artificial
  Synthetic construct
QDISNYLN

SEQ ID NO: 32 - protein, 7 aa, Artificial
  Synthetic construct
FTSSLHS

SEQ ID NO: 33 - protein, 9 aa, Artificial
  Synthetic construct
QQYSTVPWT

SEQ ID NO: 34 - protein, 123 aa, Artificial
  Synthetic construct
EVQLVESGGGLVQPGGSLRLSCAASGYDFTHYGMNWVRQAPGKCLEWVGWINTYTGEPTYAADFKRRFTFSLDTSKSTAYLQMNSLRAEDTAVYYCAKYPYYYGTSHWYFDVWGQGTLVTVSS

SEQ ID NO: 35 - protein, 7 aa, Artificial
  Synthetic construct
GYDFTHY

SEQ ID NO: 36 - protein, 6 aa, Artificial
  Synthetic construct
NTYTGE

SEQ ID NO: 37 - protein, 14 aa, Artificial
  Synthetic construct
YPYYYGTSHWYFDV

SEQ ID NO: 38 - protein, 449 aa, Artificial
  Synthetic construct
EVRLLESGGGLVQPGGSLRLSCAASGFTFSNYAMGWVRQAPGKGLEWVSAISGSGGSTYYADSVKGRFTTSRDDSKNALYLQMNSLRAEDTAVYYCARGGPGWYAADVWGQGTTVTVSSASTKGPSVFPLAPSSKSTSGGTAALGCLVKDYFPEPVTVSWNSGALTSGVHTFPAVLQSSGLYSLSSVVTVPSSSLGTQTYICNVNHKPSNTKVDKKAEPKSCDKTHTCPPCPAPELLGGPSVFLFPPKPKDTLMISRTPEVTCVVVDVSHEDPEVKFNWYVDGVEVHNAKTKPREEQYNSTYRVVSVLTVLHQDWLNGKEYKCKVSNKALPAPIEKTISKAKGQPREPQVYTLPPSRDELTKNQVSLTCLVKGFYPSDIAVEWESNGQPENNYKTTPPVLDSDGSFFLYSKLTVDKSRWQQGNVFSCSVMHEALHNHYTQKSLSLSPGK

SEQ ID NO: 39 - protein, 125 aa, Artificial; identical to SEQ ID NO: 12
  Synthetic construct

SEQ ID NO: 40 - protein, 214 aa, Artificial
  Synthetic construct
DIQLTQSPSSLSASVGDRVTITCSASQDISNYLNWYQQKPGKAPKVLIYFTSSLHSGVPSRFSGSGSGTDFTLTISSLQPEDFATYYCQQYSTVPWTFGQGTKVEIKRTVAAPSVFIFPPSDEQLKSGTASVVCLLNNFYPREAKVQWKVDNALQSGNSQESVTEQDSKDSTYSLSSTLTLSKADYEKHKVYACEVTHQGLSSPVTKSFNRGEC

SEQ ID NO: 41 - protein, 213 aa, Artificial
  Synthetic construct
SYVLTQPPSVSVAPGQTARITCGGNNIGSKSVHWYQQKPGQAPVLVVYDDSDRPSGIPERFSGSNSGNTATLTISRVEAGDEADYYCQVWDSSSDHWVFGGGTKLTVLSSASTKGPSVFPLAPSSKSTSGGTAALGCLVKDYFPEPVTVSWNSGALTSGVHTFPAVLQSSGLYSLSSVVTVPSSSLGTQTYICNVNHKPSNTKVDKKVEPKSC

SEQ ID NO: 42 - protein, 214 aa, Artificial
  Synthetic construct
DIQMTQSPSSLSASVGDRVTITCRASQSISSYLNWYQQKPGKAPKLLIYAASSLQSGVPSRFSGSGSGTDFTLTISSLQPEDFATYYCQQADLPAFAFGGGTKVEIKRTVAAPSVFIFPPSDEQLKSGTASVVCLLNNFYPREAKVQWKVDNALQSGNSQESVTEQDSKDSTYSLSSTLTLSKADYEKHKVYACEVTHQGLSSPVTKSFNRGEC